European Patent Application EP 4 424 699 A1, published September 4, 2024. Title: HBV core protein binding compounds and uses thereof. Applicant: Julius-Maximilians-Universität Würzburg. Application EP. The sequence listing filed with the application follows.

SEQUENCE LISTING (25 sequences)

SEQ ID NO: 1 - skipped

SEQ ID NO: 2 - protein, 6 aa, synthetic construct
  VARIANT 6: note = is selected from methionine (M), valine (V), leucine (L), isoleucine (I), phenylalanine (F), and non-natural amino acids comprising hydrophobic exchange(s)
SLLGRX

SEQ ID NO: 3 - protein, 10 aa, synthetic construct
  PEPTIDE 7
  VARIANT 7: note = is selected from methionine (M), valine (V), leucine (L), isoleucine (I), phenylalanine (F), and non-natural amino acids comprising hydrophobic exchange(s)
GSLLGRXKGA

SEQ ID NO: 4 - protein, 12 aa, synthetic construct
  VARIANT 11: note = is selected from methionine (M), valine (V), leucine (L), isoleucine (I), phenylalanine (F), and non-natural amino acids comprising hydrophobic exchange(s)
MHRSLLGRXKGA

SEQ ID NO: 5 - protein, 6 aa, synthetic construct
SLLGRM

SEQ ID NO: 6 - protein, 6 aa, synthetic construct
SLLGRL

SEQ ID NO: 7 - protein, 6 aa, synthetic construct
SLLGRI

SEQ ID NO: 8 - protein, 6 aa, synthetic construct
SLLGRV

SEQ ID NO: 9 - protein, 6 aa, synthetic construct
SLLGRF

SEQ ID NO: 10 - protein, 10 aa, synthetic construct
GSLLGRMKGA

SEQ ID NO: 11 - protein, 10 aa, synthetic construct
GSLLGRLKGA

SEQ ID NO: 12 - protein, 10 aa, synthetic construct
GSLLGRIKGA

SEQ ID NO: 13 - protein, 10 aa, synthetic construct
GSLLGRVKGA

SEQ ID NO: 14 - protein, 10 aa, synthetic construct
GSLLGRFKGA

SEQ ID NO: 15 - protein, 12 aa, synthetic construct
MHRSLLGRMKGA

SEQ ID NO: 16 - protein, 12 aa, synthetic construct
MHRSLLGRLKGA

SEQ ID NO: 17 - protein, 12 aa, synthetic construct
MHRSLLGRIKGA

SEQ ID NO: 18 - protein, 12 aa, synthetic construct
MHRSLLGRVKGA

SEQ ID NO: 19 - protein, 12 aa, synthetic construct
MHRSLLGRFKGA

SEQ ID NO: 20 - protein, 6 aa, synthetic construct
LLGRMK

SEQ ID NO: 21 - protein, 8 aa, synthetic construct
ALLGRMKG

SEQ ID NO: 22 - protein, 9 aa, synthetic construct
SLLGRMKGA

SEQ ID NO: 23 - protein, 8 aa, synthetic construct
SLLGRMKG

SEQ ID NO: 24 - protein, 10 aa, synthetic construct
RRRRRRRRRR

SEQ ID NO: 25 - protein, 211 aa, Hepatitis B virus
MQLFHLCLIISCSCPTVQASKLCLGWLWGMDIDPYKEFGATVELSFLPSDFFPSVRDLLDTASALYREALESPEHCSPHHTALRQAILCWGELMTLATWVGVNLEDPASRDLVVSYVNTNMGLKFRQLLWFHISCLTFGRETVIEYLVSFGVWIRTPPAYRPPNAPILSTLPETTVVRRRGRSPRRRTPSPRRRRSQSPRRRRSQSRESQC